European Patent Specification EP 3 914 720 B9, published September 27, 2023. Title: VGLL4 WITH UCP-1 CIS-REGULATORY ELEMENT AND METHOD OF USE THEREOF. Applicant: MASONIC MEDIACL RESEARCH INSTITUTE. The sequence listing filed with the application follows.

SEQUENCE LISTING (44 sequences)

SEQ ID NO: 1 - DNA, 638 bp, Mus musculus
gcatgccaatttatagtgccgtcactaacagtactgatactttaacatgctaagtttaaagtgtgtgctatattaattgtaagattggtgaagagaggtgttatcagatggaagctgcacatttctggattaatgtggttaaatgtatcttctcctgtgattactgtctttatttcttcttttaaaatattgtcatttggacatctatctgtatagctacgccctgacacgtcctcctggagacagataagaagttacgacgggaggagcagatggaggcaaagcgctgtgatgcttttgtggtttgagtgcacacatttgttcagtgattctgtgaaatgagtgagcaaatggtgaccgggtgccctgtaaatggtgttctacatcttaagagaagaacacggacactaggtaagtgaagcttgctgtcactcctctacagcgtcacagagggtcagtcacccttgaccacactgaactagtcgtcacctttccactcttcctgccagaagagcagaaatcagactctctggggatatcagcctcacccctactgctctctccattatgaggcaaactttctttcacttcccagaggctctgggggcagcaaggtcaaccctttcctcagactctag

SEQ ID NO: 2 - DNA, 335 bp, Mus musculus
tctcggaggagatcagatcgcgcttattcaagggaaccagcccctgctctgcgccctggtccaaggctgttgaagagtgacaaaaggcaccacgctgcggggacgcgggtgaagcccctctgtgtgtcctctgggcataatcaggaactggtgccaaatcagaggtgatgtggccagggctttgggagtgacgcgcggctgggaggcttgcgcacccaaggcacgcccctgccaagtcccactagcagctctttggagacctgggccggctcagccacttcccccagtccctcctccggcaaggggctatatagatctcccaggtcagggcgcag

SEQ ID NO: 3 - DNA, 973 bp, Artificial Sequence
  Laboratory-synthesized seqeunce.
gcatgccaatttatagtgccgtcactaacagtactgatactttaacatgctaagtttaaagtgtgtgctatattaattgtaagattggtgaagagaggtgttatcagatggaagctgcacatttctggattaatgtggttaaatgtatcttctcctgtgattactgtctttatttcttcttttaaaatattgtcatttggacatctatctgtatagctacgccctgacacgtcctcctggagacagataagaagttacgacgggaggagcagatggaggcaaagcgctgtgatgcttttgtggtttgagtgcacacatttgttcagtgattctgtgaaatgagtgagcaaatggtgaccgggtgccctgtaaatggtgttctacatcttaagagaagaacacggacactaggtaagtgaagcttgctgtcactcctctacagcgtcacagagggtcagtcacccttgaccacactgaactagtcgtcacctttccactcttcctgccagaagagcagaaatcagactctctggggatatcagcctcacccctactgctctctccattatgaggcaaactttctttcacttcccagaggctctgggggcagcaaggtcaaccctttcctcagactctagtctcggaggagatcagatcgcgcttattcaagggaaccagcccctgctctgcgccctggtccaaggctgttgaagagtgacaaaaggcaccacgctgcggggacgcgggtgaagcccctctgtgtgtcctctgggcataatcaggaactggtgccaaatcagaggtgatgtggccagggctttgggagtgacgcgcggctgggaggcttgcgcacccaaggcacgcccctgccaagtcccactagcagctctttggagacctgggccggctcagccacttcccccagtccctcctccggcaaggggctatatagatctcccaggtcagggcgcag

SEQ ID NO: 4 - DNA, 295 bp, Rattus norvegicus
gacgtcacagtgggtcagtcacccttgatcacactgcaccagtcttcacctttccacgcttcctgccagagcatgaatcaggctctctggggataccggcctcacccctactgaggcaaactttctcccacttctcagaggctctgagggcagcaaggtcagccctttctttggaatctagaaccactccctgtcttgagctgacatcacagggcaggcagatgcagcagggaagggcctgggactgggacgttcatcctacaagaaagctgtggaacttttcagcaacatctca

SEQ ID NO: 5 - DNA, 427 bp, Rattus norvegicus
gaaatcagatcgcacttattcaaaggagccaggccctgctctgcgccctggtggaggctcctcatgtgaagagtgacaaaaggcaccatgttgtggatacggggcgaagcccctccggtgtgtcctccaggcatcatcaggaactagtgccaaagcagaggtgctggccagggctttgggagtgacgcgcgtctgggaggcttgtgcgcccagggcacgcccctgccgattcccactagcaggtcttgggggacctgggccggctctgcccctcctccagcaatcgggctataaagctcttccaagtcagggcgcagaagtgccgggcgatccgggcttaaagagcgagaggaagggacgctcacctttgagctcctccacaaatagccctggtggctgccacagaagttcgaagttgagagttcgg

SEQ ID NO: 6 - DNA, 722 bp, Artificial Sequence
  Laboratory-synthesized seqeunce
gacgtcacagtgggtcagtcacccttgatcacactgcaccagtcttcacctttccacgcttcctgccagagcatgaatcaggctctctggggataccggcctcacccctactgaggcaaactttctcccacttctcagaggctctgagggcagcaaggtcagccctttctttggaatctagaaccactccctgtcttgagctgacatcacagggcaggcagatgcagcagggaagggcctgggactgggacgttcatcctacaagaaagctgtggaacttttcagcaacatctcagaaatcagatcgcacttattcaaaggagccaggccctgctctgcgccctggtggaggctcctcatgtgaagagtgacaaaaggcaccatgttgtggatacggggcgaagcccctccggtgtgtcctccaggcatcatcaggaactagtgccaaagcagaggtgctggccagggctttgggagtgacgcgcgtctgggaggcttgtgcgcccagggcacgcccctgccgattcccactagcaggtcttgggggacctgggccggctctgcccctcctccagcaatcgggctataaagctcttccaagtcagggcgcagaagtgccgggcgatccgggcttaaagagcgagaggaagggacgctcacctttgagctcctccacaaatagccctggtggctgccacagaagttcgaagttgagagttcgg

SEQ ID NO: 7 - DNA, 334 bp, Homo sapiens
tgatcaagtgcatttgttaatgtgttctacattttcaaaaaggaaaggagaatttgttacattcagaacttgctgccactcctttgctacgtcataaagggtcagttgcccttgctcatactgacctattctttacctctctgcttcttctttgtgccagaagagtagaaatctgaccctttggggataccaccctctcccctactgctctctccaacctgaggcaaactttctcctacttcccagagcctgtcagaagtggtgaagccagcctgctccttggaatccagaactactttcagaatcttgaacttctgtgacctctcagggtccc

SEQ ID NO: 8 - DNA, 289 bp, Homo sapiens
accgccgcggtgcgccctccctccgacgtgcggtgtgcggggcgcagacaaccagcggccggcccagggctttcggggagcgaagcagggctcccgaggcaccgagcgagaatgggaatgggagggacccggtgctcccggacacgcccccggcaggtcccacgcccgggtcttctgagacctcgcgcggcccagcccgggagcggcccagctatataagtcccagcggaagaccggaacgcagagggtcctgctggcgcgagggtgggtaggaggggacgcggggact

SEQ ID NO: 9 - DNA, 623 bp, Homo sapiens
tgatcaagtgcatttgttaatgtgttctacattttcaaaaaggaaaggagaatttgttacattcagaacttgctgccactcctttgctacgtcataaagggtcagttgcccttgctcatactgacctattctttacctctctgcttcttctttgtgccagaagagtagaaatctgaccctttggggataccaccctctcccctactgctctctccaacctgaggcaaactttctcctacttcccagagcctgtcagaagtggtgaagccagcctgctccttggaatccagaactactttcagaatcttgaacttctgtgacctctcagggtcccaccgccgcggtgcgccctccctccgacgtgcggtgtgcggggcgcagacaaccagcggccggcccagggctttcggggagcgaagcagggctcccgaggcaccgagcgagaatgggaatgggagggacccggtgctcccggacacgcccccggcaggtcccacgcccgggtcttctgagacctcgcgcggcccagcccgggagcggcccagctatataagtcccagcggaagaccggaacgcagagggtcctgctggcgcgagggtgggtaggaggggacgcggggact

SEQ ID NO: 10 - DNA, 888 bp, Homo sapiens
atgctatttatgaagatggacctgttgaactatcagtacttggacaagatgaacaacaatatcggcattctgtgctacgaaggcgaagctgctctcaggggagaacccagaatacagaccctgccggtggcctctgccctcagcagtcaccgcaccggccctcccccaatcagccccagcaagaggaagttcagcatggagccaggtgacgaggacctagactgtgacaacgaccacgtctccaaaatgagtcgcatcttcaacccccatctgaacaagactgccaatggagactgccgcagagacccccgggagcggagccgcagccccatcgagcgcgctgtggcccccaccatgagcctgcacggcagccacctgtacacctccctccccagccttggcctggagcagcccctcgcactgaccaagaacagcctggacgccagcaggccagccggcctctcgcccacactgaccccgggggagcggcagcagaaccggccctccgtgatcacctgtgcctcggctggcgcccgcaactgcaacctctcgcactgccccatcgcgcacagcggctgtgccgcgcccgggcctgccagctaccggaggccaccgagcgctgccaccacctgtgaccccgtggtggaggagcatttccgcaggagcctgggcaagaattacaaggagcccgagccggcacccaactccgtgtccatcacgggctccgtggacgaccactttgccaaagctctgggtgacacgtggctccagatcaaagcggccaaggacggagcatccagcagccctgagtccgcctctcgcaggggccagcccgccagcccctctgcccacatggtcagccacagtcactccccctctgtggtctcc

SEQ ID NO: 11 - protein, 296 aa, Homo sapiens
MLFMKMDLLNYQYLDKMNNNIGILCYEGEAALRGEPRIQTLPVASALSSHRTGPPPISPSKRKFSMEPGDEDLDCDNDHVSKMSRIFNPHLNKTANGDCRRDPRERSRSPIERAVAPTMSLHGSHLYTSLPSLGLEQPLALTKNSLDASRPAGLSPTLTPGERQQNRPSVITCASAGARNCNLSHCPIAHSGCAAPGPASYRRPPSAATTCDPVVEEHFRRSLGKNYKEPEPAPNSVSITGSVDDHFAKALGDTWLQIKAAKDGASSSPESASRRGQPASPSAHMVSHSHSPSVVS

SEQ ID NO: 12 - DNA, 870 bp, Homo sapiens
atggagacgccattggatgttttgtccagggcagcatctctggtgcatgctgatgacgaaaaacgcgaagctgctctcaggggagaacccagaatacagaccctgccggtggcctctgccctcagcagtcaccgcaccggccctcccccaatcagccccagcaagaggaagttcagcatggagccaggtgacgaggacctagactgtgacaacgaccacgtctccaaaatgagtcgcatcttcaacccccatctgaacaagactgccaatggagactgccgcagagacccccgggagcggagccgcagccccatcgagcgcgctgtggcccccaccatgagcctgcacggcagccacctgtacacctccctccccagccttggcctggagcagcccctcgcactgaccaagaacagcctggacgccagcaggccagccggcctctcgcccacactgaccccgggggagcggcagcagaaccggccctccgtgatcacctgtgcctcggctggcgcccgcaactgcaacctctcgcactgccccatcgcgcacagcggctgtgccgcgcccgggcctgccagctaccggaggccaccgagcgctgccaccacctgtgaccccgtggtggaggagcatttccgcaggagcctgggcaagaattacaaggagcccgagccggcacccaactccgtgtccatcacgggctccgtggacgaccactttgccaaagctctgggtgacacgtggctccagatcaaagcggccaaggacggagcatccagcagccctgagtccgcctctcgcaggggccagcccgccagcccctctgcccacatggtcagccacagtcactccccctctgtggtctcc

SEQ ID NO: 13 - protein, 290 aa, Homo sapiens
METPLDVLSRAASLVHADDEKREAALRGEPRIQTLPVASALSSHRTGPPPISPSKRKFSMEPGDEDLDCDNDHVSKMSRIFNPHLNKTANGDCRRDPRERSRSPIERAVAPTMSLHGSHLYTSLPSLGLEQPLALTKNSLDASRPAGLSPTLTPGERQQNRPSVITCASAGARNCNLSHCPIAHSGCAAPGPASYRRPPSAATTCDPVVEEHFRRSLGKNYKEPEPAPNSVSITGSVDDHFAKALGDTWLQIKAAKDGASSSPESASRRGQPASPSAHMVSHSHSPSVVS

SEQ ID NO: 14 - DNA, 630 bp, Homo sapiens
atgattaaagtgaggaacaagactgccaatggagactgccgcagagacccccgggagcggagccgcagccccatcgagcgcgctgtggcccccaccatgagcctgcacggcagccacctgtacacctccctccccagccttggcctggagcagcccctcgcactgaccaagaacagcctggacgccagcaggccagccggcctctcgcccacactgaccccgggggagcggcagcagaaccggccctccgtgatcacctgtgcctcggctggcgcccgcaactgcaacctctcgcactgccccatcgcgcacagcggctgtgccgcgcccgggcctgccagctaccggaggccaccgagcgctgccaccacctgtgaccccgtggtggaggagcatttccgcaggagcctgggcaagaattacaaggagcccgagccggcacccaactccgtgtccatcacgggctccgtggacgaccactttgccaaagctctgggtgacacgtggctccagatcaaagcggccaaggacggagcatccagcagccctgagtccgcctctcgcaggggccagcccgccagcccctctgcccacatggtcagccacagtcactccccctctgtggtctcc

SEQ ID NO: 15 - protein, 210 aa, Homo sapiens
MIKVRNKTANGDCRRDPRERSRSPIERAVAPTMSLHGSHLYTSLPSLGLEQPLALTKNSLDASRPAGLSPTLTPGERQQNRPSVITCASAGARNCNLSHCPIAHSGCAAPGPASYRRPPSAATTCDPVVEEHFRRSLGKNYKEPEPAPNSVSITGSVDDHFAKALGDTWLQIKAAKDGASSSPESASRRGQPASPSAHMVSHSHSPSVVS

SEQ ID NO: 16 - DNA, 618 bp, Homo sapiens
atgaacaagactgccaatggagactgccgcagagacccccgggagcggagccgcagccccatcgagcgcgctgtggcccccaccatgagcctgcacggcagccacctgtacacctccctccccagccttggcctggagcagcccctcgcactgaccaagaacagcctggacgccagcaggccagccggcctctcgcccacactgaccccgggggagcggcagcagaaccggccctccgtgatcacctgtgcctcggctggcgcccgcaactgcaacctctcgcactgccccatcgcgcacagcggctgtgccgcgcccgggcctgccagctaccggaggccaccgagcgctgccaccacctgtgaccccgtggtggaggagcatttccgcaggagcctgggcaagaattacaaggagcccgagccggcacccaactccgtgtccatcacgggctccgtggacgaccactttgccaaagctctgggtgacacgtggctccagatcaaagcggccaaggacggagcatccagcagccctgagtccgcctctcgcaggggccagcccgccagcccctctgcccacatggtcagccacagtcactccccctctgtggtctcc

SEQ ID NO: 17 - protein, 206 aa, Homo sapiens
MNKTANGDCRRDPRERSRSPIERAVAPTMSLHGSHLYTSLPSLGLEQPLALTKNSLDASRPAGLSPTLTPGERQQNRPSVITCASAGARNCNLSHCPIAHSGCAAPGPASYRRPPSAATTCDPVVEEHFRRSLGKNYKEPEPAPNSVSITGSVDDHFAKALGDTWLQIKAAKDGASSSPESASRRGQPASPSAHMVSHSHSPSVVS

SEQ ID NO: 18 - DNA, 885 bp, Homo sapiens
atgactgagaatacgcattttgacaaaatccctgagtcctgtgcactcaaaagttggagacatccaggtctgcaccatggcgaagctgctctcaggggagaacccagaatacagaccctgccggtggcctctgccctcagcagtcaccgcaccggccctcccccaatcagccccagcaagaggaagttcagcatggagccaggtgacgaggacctagactgtgacaacgaccacgtctccaaaatgagtcgcatcttcaacccccatctgaacaagactgccaatggagactgccgcagagacccccgggagcggagccgcagccccatcgagcgcgctgtggcccccaccatgagcctgcacggcagccacctgtacacctccctccccagccttggcctggagcagcccctcgcactgaccaagaacagcctggacgccagcaggccagccggcctctcgcccacactgaccccgggggagcggcagcagaaccggccctccgtgatcacctgtgcctcggctggcgcccgcaactgcaacctctcgcactgccccatcgcgcacagcggctgtgccgcgcccgggcctgccagctaccggaggccaccgagcgctgccaccacctgtgaccccgtggtggaggagcatttccgcaggagcctgggcaagaattacaaggagcccgagccggcacccaactccgtgtccatcacgggctccgtggacgaccactttgccaaagctctgggtgacacgtggctccagatcaaagcggccaaggacggagcatccagcagccctgagtccgcctctcgcaggggccagcccgccagcccctctgcccacatggtcagccacagtcactccccctctgtggtctcc

SEQ ID NO: 19 - protein, 295 aa, Homo sapiens
MTENTHFDKIPESCALKSWRHPGLHHGEAALRGEPRIQTLPVASALSSHRTGPPPISPSKRKFSMEPGDEDLDCDNDHVSKMSRIFNPHLNKTANGDCRRDPRERSRSPIERAVAPTMSLHGSHLYTSLPSLGLEQPLALTKNSLDASRPAGLSPTLTPGERQQNRPSVITCASAGARNCNLSHCPIAHSGCAAPGPASYRRPPSAATTCDPVVEEHFRRSLGKNYKEPEPAPNSVSITGSVDDHFAKALGDTWLQIKAAKDGASSSPESASRRGQPASPSAHMVSHSHSPSVVS

SEQ ID NO: 20 - DNA, 693 bp, Homo sapiens
atggagccaggtgacgaggacctagactgtgacaacgaccacgtctccaaaatgagtcgcatcttcaacccccatctgaacaagactgccaatggagactgccgcagagacccccgggagcggagccgcagccccatcgagcgcgctgtggcccccaccatgagcctgcacggcagccacctgtacacctccctccccagccttggcctggagcagcccctcgcactgaccaagaacagcctggacgccagcaggccagccggcctctcgcccacactgaccccgggggagcggcagcagaaccggccctccgtgatcacctgtgcctcggctggcgcccgcaactgcaacctctcgcactgccccatcgcgcacagcggctgtgccgcgcccgggcctgccagctaccggaggccaccgagcgctgccaccacctgtgaccccgtggtggaggagcatttccgcaggagcctgggcaagaattacaaggagcccgagccggcacccaactccgtgtccatcacgggctccgtggacgaccactttgccaaagctctgggtgacacgtggctccagatcaaagcggccaaggacggagcatccagcagccctgagtccgcctctcgcaggggccagcccgccagcccctctgcccacatggtcagccacagtcactccccctctgtggtctcc

SEQ ID NO: 21 - protein, 231 aa, Homo sapiens
MEPGDEDLDCDNDHVSKMSRIFNPHLNKTANGDCRRDPRERSRSPIERAVAPTMSLHGSHLYTSLPSLGLEQPLALTKNSLDASRPAGLSPTLTPGERQQNRPSVITCASAGARNCNLSHCPIAHSGCAAPGPASYRRPPSAATTCDPVVEEHFRRSLGKNYKEPEPAPNSVSITGSVDDHFAKALGDTWLQIKAAKDGASSSPESASRRGQPASPSAHMVSHSHSPSVVS

SEQ ID NO: 22 - DNA, 888 bp, Artificial Sequence
  Laboratory-synthesized seqeunce
atgctatttatgaagatggacctgttgaactatcagtacttggacaagatgaacaacaatatcggcattctgtgctacgaaggcgaagctgctctcaggggagaacccagaatacagaccctgccggtggcctctgccctcagcagtcaccgcaccggccctcccccaatcagccccagcaagaggaagttcagcatggagccaggtgacgaggacctagactgtgacaacgaccacgtctccaaaatgagtcgcatcttcaacccccatctgaacaagactgccaatggagactgccgcagagacccccgggagcggagccgcagccccatcgagcgcgctgtggcccccaccatgagcctgcacggcagccacctgtacacctccctccccagccttggcctggagcagcccctcgcactgaccaagaacagcctggacgccagcaggccagccggcctctcgcccacactgaccccgggggagcggcagcagaaccggccctccgtgatcacctgtgcctcggctggcgcccgcaactgcaacctctcgcactgccccatcgcgcacagcggctgtgccgcgcccgggcctgccagctaccggaggccaccgagcgctgccaccacctgtgaccccgtggtggaggaggcagcccgcaggagcctgggcaagaattacaaggagcccgagccggcacccaactccgtgtccatcacgggctccgtggacgacgcagctgccaaagctctgggtgacacgtggctccagatcaaagcggccaaggacggagcatccagcagccctgagtccgcctctcgcaggggccagcccgccagcccctctgcccacatggtcagccacagtcactccccctctgtggtctcc

SEQ ID NO: 23 - protein, 296 aa, Artificial Sequence
  Laboratory-synthesized seqeunce
MLFMKMDLLNYQYLDKMNNNIGILCYEGEAALRGEPRIQTLPVASALSSHRTGPPPISPSKRKFSMEPGDEDLDCDNDHVSKMSRIFNPHLNKTANGDCRRDPRERSRSPIERAVAPTMSLHGSHLYTSLPSLGLEQPLALTKNSLDASRPAGLSPTLTPGERQQNRPSVITCASAGARNCNLSHCPIAHSGCAAPGPASYRRPPSAATTCDPVVEEAARRSLGKNYKEPEPAPNSVSITGSVDDAAAKALGDTWLQIKAAKDGASSSPESASRRGQPASPSAHMVSHSHSPSVVS

SEQ ID NO: 24 - DNA, 870 bp, Artificial Sequence
  Laboratory-synthesized seqeunce
atggagacgccattggatgttttgtccagggcagcatctctggtgcatgctgatgacgaaaaacgcgaagctgctctcaggggagaacccagaatacagaccctgccggtggcctctgccctcagcagtcaccgcaccggccctcccccaatcagccccagcaagaggaagttcagcatggagccaggtgacgaggacctagactgtgacaacgaccacgtctccaaaatgagtcgcatcttcaacccccatctgaacaagactgccaatggagactgccgcagagacccccgggagcggagccgcagccccatcgagcgcgctgtggcccccaccatgagcctgcacggcagccacctgtacacctccctccccagccttggcctggagcagcccctcgcactgaccaagaacagcctggacgccagcaggccagccggcctctcgcccacactgaccccgggggagcggcagcagaaccggccctccgtgatcacctgtgcctcggctggcgcccgcaactgcaacctctcgcactgccccatcgcgcacagcggctgtgccgcgcccgggcctgccagctaccggaggccaccgagcgctgccaccacctgtgaccccgtggtggaggaggcagcccgcaggagcctgggcaagaattacaaggagcccgagccggcacccaactccgtgtccatcacgggctccgtggacgacgcagctgccaaagctctgggtgacacgtggctccagatcaaagcggccaaggacggagcatccagcagccctgagtccgcctctcgcaggggccagcccgccagcccctctgcccacatggtcagccacagtcactccccctctgtggtctcc

SEQ ID NO: 25 - protein, 290 aa, Artificial Sequence
  Laboratory-synthesized seqeunce
METPLDVLSRAASLVHADDEKREAALRGEPRIQTLPVASALSSHRTGPPPISPSKRKFSMEPGDEDLDCDNDHVSKMSRIFNPHLNKTANGDCRRDPRERSRSPIERAVAPTMSLHGSHLYTSLPSLGLEQPLALTKNSLDASRPAGLSPTLTPGERQQNRPSVITCASAGARNCNLSHCPIAHSGCAAPGPASYRRPPSAATTCDPVVEEAARRSLGKNYKEPEPAPNSVSITGSVDDAAAKALGDTWLQIKAAKDGASSSPESASRRGQPASPSAHMVSHSHSPSVVS

SEQ ID NO: 26 - DNA, 630 bp, Artificial Sequence
  Laboratory-synthesized seqeunce
atgattaaagtgaggaacaagactgccaatggagactgccgcagagacccccgggagcggagccgcagccccatcgagcgcgctgtggcccccaccatgagcctgcacggcagccacctgtacacctccctccccagccttggcctggagcagcccctcgcactgaccaagaacagcctggacgccagcaggccagccggcctctcgcccacactgaccccgggggagcggcagcagaaccggccctccgtgatcacctgtgcctcggctggcgcccgcaactgcaacctctcgcactgccccatcgcgcacagcggctgtgccgcgcccgggcctgccagctaccggaggccaccgagcgctgccaccacctgtgaccccgtggtggaggaggcagcccgcaggagcctgggcaagaattacaaggagcccgagccggcacccaactccgtgtccatcacgggctccgtggacgacgcagctgccaaagctctgggtgacacgtggctccagatcaaagcggccaaggacggagcatccagcagccctgagtccgcctctcgcaggggccagcccgccagcccctctgcccacatggtcagccacagtcactccccctctgtggtctcc

SEQ ID NO: 27 - protein, 210 aa, Artificial Sequence
  Laboratory-synthesized seqeunce
MIKVRNKTANGDCRRDPRERSRSPIERAVAPTMSLHGSHLYTSLPSLGLEQPLALTKNSLDASRPAGLSPTLTPGERQQNRPSVITCASAGARNCNLSHCPIAHSGCAAPGPASYRRPPSAATTCDPVVEEAARRSLGKNYKEPEPAPNSVSITGSVDDAAAKALGDTWLQIKAAKDGASSSPESASRRGQPASPSAHMVSHSHSPSVVS

SEQ ID NO: 28 - DNA, 618 bp, Artificial Sequence
  Laboratory-synthesized seqeunce
atgaacaagactgccaatggagactgccgcagagacccccgggagcggagccgcagccccatcgagcgcgctgtggcccccaccatgagcctgcacggcagccacctgtacacctccctccccagccttggcctggagcagcccctcgcactgaccaagaacagcctggacgccagcaggccagccggcctctcgcccacactgaccccgggggagcggcagcagaaccggccctccgtgatcacctgtgcctcggctggcgcccgcaactgcaacctctcgcactgccccatcgcgcacagcggctgtgccgcgcccgggcctgccagctaccggaggccaccgagcgctgccaccacctgtgaccccgtggtggaggaggcagcccgcaggagcctgggcaagaattacaaggagcccgagccggcacccaactccgtgtccatcacgggctccgtggacgacgcagctgccaaagctctgggtgacacgtggctccagatcaaagcggccaaggacggagcatccagcagccctgagtccgcctctcgcaggggccagcccgccagcccctctgcccacatggtcagccacagtcactccccctctgtggtctcc

SEQ ID NO: 29 - protein, 206 aa, Artificial Sequence
  Laboratory-synthesized seqeunce
MNKTANGDCRRDPRERSRSPIERAVAPTMSLHGSHLYTSLPSLGLEQPLALTKNSLDASRPAGLSPTLTPGERQQNRPSVITCASAGARNCNLSHCPIAHSGCAAPGPASYRRPPSAATTCDPVVEEAARRSLGKNYKEPEPAPNSVSITGSVDDAAAKALGDTWLQIKAAKDGASSSPESASRRGQPASPSAHMVSHSHSPSVVS

SEQ ID NO: 30 - DNA, 885 bp, Artificial Sequence
  Laboratory-synthesized seqeunce
atgactgagaatacgcattttgacaaaatccctgagtcctgtgcactcaaaagttggagacatccaggtctgcaccatggcgaagctgctctcaggggagaacccagaatacagaccctgccggtggcctctgccctcagcagtcaccgcaccggccctcccccaatcagccccagcaagaggaagttcagcatggagccaggtgacgaggacctagactgtgacaacgaccacgtctccaaaatgagtcgcatcttcaacccccatctgaacaagactgccaatggagactgccgcagagacccccgggagcggagccgcagccccatcgagcgcgctgtggcccccaccatgagcctgcacggcagccacctgtacacctccctccccagccttggcctggagcagcccctcgcactgaccaagaacagcctggacgccagcaggccagccggcctctcgcccacactgaccccgggggagcggcagcagaaccggccctccgtgatcacctgtgcctcggctggcgcccgcaactgcaacctctcgcactgccccatcgcgcacagcggctgtgccgcgcccgggcctgccagctaccggaggccaccgagcgctgccaccacctgtgaccccgtggtggaggaggcagcccgcaggagcctgggcaagaattacaaggagcccgagccggcacccaactccgtgtccatcacgggctccgtggacgacgcagctgccaaagctctgggtgacacgtggctccagatcaaagcggccaaggacggagcatccagcagccctgagtccgcctctcgcaggggccagcccgccagcccctctgcccacatggtcagccacagtcactccccctctgtggtctcc

SEQ ID NO: 31 - protein, 295 aa, Artificial Sequence
  Laboratory-synthesized seqeunce
MTENTHFDKIPESCALKSWRHPGLHHGEAALRGEPRIQTLPVASALSSHRTGPPPISPSKRKFSMEPGDEDLDCDNDHVSKMSRIFNPHLNKTANGDCRRDPRERSRSPIERAVAPTMSLHGSHLYTSLPSLGLEQPLALTKNSLDASRPAGLSPTLTPGERQQNRPSVITCASAGARNCNLSHCPIAHSGCAAPGPASYRRPPSAATTCDPVVEEAARRSLGKNYKEPEPAPNSVSITGSVDDAAAKALGDTWLQIKAAKDGASSSPESASRRGQPASPSAHMVSHSHSPSVVS

SEQ ID NO: 32 - DNA, 693 bp, Artificial Sequence
  Laboratory-synthesized seqeunce
atggagccaggtgacgaggacctagactgtgacaacgaccacgtctccaaaatgagtcgcatcttcaacccccatctgaacaagactgccaatggagactgccgcagagacccccgggagcggagccgcagccccatcgagcgcgctgtggcccccaccatgagcctgcacggcagccacctgtacacctccctccccagccttggcctggagcagcccctcgcactgaccaagaacagcctggacgccagcaggccagccggcctctcgcccacactgaccccgggggagcggcagcagaaccggccctccgtgatcacctgtgcctcggctggcgcccgcaactgcaacctctcgcactgccccatcgcgcacagcggctgtgccgcgcccgggcctgccagctaccggaggccaccgagcgctgccaccacctgtgaccccgtggtggaggaggcagcccgcaggagcctgggcaagaattacaaggagcccgagccggcacccaactccgtgtccatcacgggctccgtggacgacgcagctgccaaagctctgggtgacacgtggctccagatcaaagcggccaaggacggagcatccagcagccctgagtccgcctctcgcaggggccagcccgccagcccctctgcccacatggtcagccacagtcactccccctctgtggtctcc

SEQ ID NO: 33 - protein, 231 aa, Artificial Sequence
  Laboratory-synthesized seqeunce
MEPGDEDLDCDNDHVSKMSRIFNPHLNKTANGDCRRDPRERSRSPIERAVAPTMSLHGSHLYTSLPSLGLEQPLALTKNSLDASRPAGLSPTLTPGERQQNRPSVITCASAGARNCNLSHCPIAHSGCAAPGPASYRRPPSAATTCDPVVEEAARRSLGKNYKEPEPAPNSVSITGSVDDAAAKALGDTWLQIKAAKDGASSSPESASRRGQPASPSAHMVSHSHSPSVVS

SEQ ID NO: 34 - DNA, 133 bp, Artificial Sequence
  Laboratory-synthesized seqeunce
gtaagtatcaaggttacaagacaggtttaaggagaccaatagaaactgggcttgtcgagacagagaagactcttgcgtttctgataggcacctattggtcttactgacatccactttgcctttctctccacag

SEQ ID NO: 35 - DNA, 2096 bp, Artificial Sequence
  Laboratory-synthesized seqeunce
gcatgccaatttatagtgccgtcactaacagtactgatactttaacatgctaagtttaaagtgtgtgctatattaattgtaagattggtgaagagaggtgttatcagatggaagctgcacatttctggattaatgtggttaaatgtatcttctcctgtgattactgtctttatttcttcttttaaaatattgtcatttggacatctatctgtatagctacgccctgacacgtcctcctggagacagataagaagttacgacgggaggagcagatggaggcaaagcgctgtgatgcttttgtggtttgagtgcacacatttgttcagtgattctgtgaaatgagtgagcaaatggtgaccgggtgccctgtaaatggtgttctacatcttaagagaagaacacggacactaggtaagtgaagcttgctgtcactcctctacagcgtcacagagggtcagtcacccttgaccacactgaactagtcgtcacctttccactcttcctgccagaagagcagaaatcagactctctggggatatcagcctcacccctactgctctctccattatgaggcaaactttctttcacttcccagaggctctgggggcagcaaggtcaaccctttcctcagactctagtctcggaggagatcagatcgcgcttattcaagggaaccagcccctgctctgcgccctggtccaaggctgttgaagagtgacaaaaggcaccacgctgcggggacgcgggtgaagcccctctgtgtgtcctctgggcataatcaggaactggtgccaaatcagaggtgatgtggccagggctttgggagtgacgcgcggctgggaggcttgcgcacccaaggcacgcccctgccaagtcccactagcagctctttggagacctgggccggctcagccacttcccccagtccctcctccggcaaggggctatatagatctcccaggtcagggcgcagctgcagaagttggtcgtgaggcactgggcaggtaagtatcaaggttacaagacaggtttaaggagaccaatagaaactgggcttgtcgagacagagaagactcttgcgtttctgataggcacctattggtcttactgacatccactttgcctttctctccacaggtgtccactcccagttcaattacagctcttaaggctagagtacttaatacgactcactataggctagcatgctatttatgaagatggacctgttgaactatcagtacttggacaagatgaacaacaatatcggcattctgtgctacgaaggcgaagctgctctcaggggagaacccagaatgcagaccctgccggtggcctctgccctcagcagtcaccgcaccggccctcccccaatcagccccagcaagaggaagttcagcatggagccaggtgacgaggacctagactgtgacaacgaccacgtctccaaaatgagtcgcatcttcaacccccatctgaacaagactgccaatggagactgccgcagagacccccgggagcggagccgcagccccatcgagcgcgctgtggcccccaccatgagcctgcacggcagccacctgtacacctccctccccagccttggcctggagcagcccctcgcactgaccaagaacagcctggacgccagcaggccagccggcctctcgcccacactgaccccgggggagcggcagcagaaccggccctccgtgatcacctgtgcctcggctggcgcccgcaactgcaacctctcgcactgccccatcgcgcacagcggctgtgccgcgcccgggcctgccagctaccggaggccaccgagcgctgccaccacctgtgaccccgtggtggaggagcatttccgcaggagcctgggcaagaattacaaggagcccgagccggcacccaactccgtgtccatcacgggctccgtggacgaccactttgccaaagctctgggtgacacgtggctccagatcaaagcggccaaggacggagcatccagcagccctgagtccgcctctcgcaggggccagcccgccagcccctctgcccacatggtcagccacagtcactccccctctgtggtctccgcc

SEQ ID NO: 36 - DNA, 2096 bp, Artificial Sequence
  Laboratory-synthesized seqeunce
gcatgccaatttatagtgccgtcactaacagtactgatactttaacatgctaagtttaaagtgtgtgctatattaattgtaagattggtgaagagaggtgttatcagatggaagctgcagcagcctggattaatgtggttaaatgtatcttctcctgtgattactgtctttatttcttcttttaaaatattgtcatttggacatctatctgtatagctacgccctgacacgtcctcctggagacagataagaagttacgacgggaggagcagatggaggcaaagcgctgtgatgcttttgtggtttgagtgcacacatttgttcagtgattctgtgaaatgagtgagcaaatggtgaccgggtgccctgtaaatggtgttctacatcttaagagaagaacacggacactaggtaagtgaagcttgctgtcactcctctacagcgtcacagagggtcagtcacccttgaccacactgaactagtcgtcacctttccactcttcctgccagaagagcagaaatcagactctctggggatatcagcctcacccctactgctctctccattatgaggcaaactttctttcacttcccagaggctctgggggcagcaaggtcaaccctttcctcagactctagtctcggaggagatcagatcgcgcttattcaagggaaccagcccctgctctgcgccctggtccaaggctgttgaagagtgacaaaaggcaccacgctgcggggacgcgggtgaagcccctctgtgtgtcctctgggcataatcaggaactggtgccaaatcagaggtgatgtggccagggctttgggagtgacgcgcggctgggaggcttgcgcacccaaggcacgcccctgccaagtcccactagcagctctttggagacctgggccggctcagccacttcccccagtccctcctccggcaaggggctatatagatctcccaggtcagggcgcagctgcagaagttggtcgtgaggcactgggcaggtaagtatcaaggttacaagacaggtttaaggagaccaatagaaactgggcttgtcgagacagagaagactcttgcgtttctgataggcacctattggtcttactgacatcgcagctgcctttctctccacaggtgtccactcccagttcaattacagctcttaaggctagagtacttaatacgactcactataggctagcatgctatttatgaagatggacctgttgaactatcagtacttggacaagatgaacaacaatatcggcattctgtgctacgaaggcgaagctgctctcaggggagaacccagaatgcagaccctgccggtggcctctgccctcagcagtcaccgcaccggccctcccccaatcagccccagcaagaggaagttcagcatggagccaggtgacgaggacctagactgtgacaacgaccacgtctccaaaatgagtcgcatcttcaacccccatctgaacaagactgccaatggagactgccgcagagacccccgggagcggagccgcagccccatcgagcgcgctgtggcccccaccatgagcctgcacggcagccacctgtacacctccctccccagccttggcctggagcagcccctcgcactgaccaagaacagcctggacgccagcaggccagccggcctctcgcccacactgaccccgggggagcggcagcagaaccggccctccgtgatcacctgtgcctcggctggcgcccgcaactgcaacctctcgcactgccccatcgcgcacagcggctgtgccgcgcccgggcctgccagctaccggaggccaccgagcgctgccaccacctgtgaccccgtggtggaggaggcagcccgcaggagcctgggcaagaattacaaggagcccgagccggcacccaactccgtgtccatcacgggctccgtggacgacgcagctgccaaagctctgggtgacacgtggctccagatcaaagcggccaaggacggagcatccagcagccctgagtccgcctctcgcaggggccagcccgccagcccctctgcccacatggtcagccacagtcactccccctctgtggtctccgcc

SEQ ID NO: 37 - protein, 239 aa, Artificial Sequence
  Laboratory-synthesized seqeunce
MVSKGEELFTGVVPILVELDGDVNGHKFSVSGEGEGDATYGKLTLKFICTTGKLPVPWPTLVTTLTYGVQCFSRYPDHMKQHDFFKSAMPEGYVQERTIFFKDDGNYKTRAEVKFEGDTLVNRIELKGIDFKEDGNILGHKLEYNYNSHNVYIMADKQKNGIKVNFKIRHNIEDGSVQLADHYQQNTPIGDGPVLLPDNHYLSTQSALSKDPNEKRDHMVLLEFVTAAGITLGMDELYK

SEQ ID NO: 38 - DNA, 720 bp, Artificial Sequence
  Laboratory-synthesized seqeunce
atggtgagcaagggcgaggagctgttcaccggggtggtgcccatcctggtcgagctggacggcgacgtaaacggccacaagttcagcgtgtccggcgagggcgagggcgatgccacctacggcaagctgaccctgaagttcatctgcaccaccggcaagctgcccgtgccctggcccaccctcgtgaccaccctgacctacggcgtgcagtgcttcagccgctaccccgaccacatgaagcagcacgacttcttcaagtccgccatgcccgaaggctacgtccaggagcgcaccatcttcttcaaggacgacggcaactacaagacccgcgccgaggtgaagttcgagggcgacaccctggtgaaccgcatcgagctgaagggcatcgacttcaaggaggacggcaacatcctggggcacaagctggagtacaactacaacagccacaacgtctatatcatggccgacaagcagaagaacggcatcaaggtgaacttcaagatccgccacaacatcgaggacggcagcgtgcagctcgccgaccactaccagcagaacacccccatcggcgacggccccgtgctgctgcccgacaaccactacctgagcacccagtccgccctgagcaaagaccccaacgagaagcgcgatcacatggtcctgctggagttcgtgaccgccgccgggatcactctcggcatggacgagctgtacaagtaa

SEQ ID NO: 39 - DNA, 2816 bp, Artificial Sequence
  Laboratory-synthesized seqeunce
gcatgccaatttatagtgccgtcactaacagtactgatactttaacatgctaagtttaaagtgtgtgctatattaattgtaagattggtgaagagaggtgttatcagatggaagctgcacatttctggattaatgtggttaaatgtatcttctcctgtgattactgtctttatttcttcttttaaaatattgtcatttggacatctatctgtatagctacgccctgacacgtcctcctggagacagataagaagttacgacgggaggagcagatggaggcaaagcgctgtgatgcttttgtggtttgagtgcacacatttgttcagtgattctgtgaaatgagtgagcaaatggtgaccgggtgccctgtaaatggtgttctacatcttaagagaagaacacggacactaggtaagtgaagcttgctgtcactcctctacagcgtcacagagggtcagtcacccttgaccacactgaactagtcgtcacctttccactcttcctgccagaagagcagaaatcagactctctggggatatcagcctcacccctactgctctctccattatgaggcaaactttctttcacttcccagaggctctgggggcagcaaggtcaaccctttcctcagactctagtctcggaggagatcagatcgcgcttattcaagggaaccagcccctgctctgcgccctggtccaaggctgttgaagagtgacaaaaggcaccacgctgcggggacgcgggtgaagcccctctgtgtgtcctctgggcataatcaggaactggtgccaaatcagaggtgatgtggccagggctttgggagtgacgcgcggctgggaggcttgcgcacccaaggcacgcccctgccaagtcccactagcagctctttggagacctgggccggctcagccacttcccccagtccctcctccggcaaggggctatatagatctcccaggtcagggcgcagctgcagaagttggtcgtgaggcactgggcaggtaagtatcaaggttacaagacaggtttaaggagaccaatagaaactgggcttgtcgagacagagaagactcttgcgtttctgataggcacctattggtcttactgacatccactttgcctttctctccacaggtgtccactcccagttcaattacagctcttaaggctagagtacttaatacgactcactataggctagcatgctatttatgaagatggacctgttgaactatcagtacttggacaagatgaacaacaatatcggcattctgtgctacgaaggcgaagctgctctcaggggagaacccagaatgcagaccctgccggtggcctctgccctcagcagtcaccgcaccggccctcccccaatcagccccagcaagaggaagttcagcatggagccaggtgacgaggacctagactgtgacaacgaccacgtctccaaaatgagtcgcatcttcaacccccatctgaacaagactgccaatggagactgccgcagagacccccgggagcggagccgcagccccatcgagcgcgctgtggcccccaccatgagcctgcacggcagccacctgtacacctccctccccagccttggcctggagcagcccctcgcactgaccaagaacagcctggacgccagcaggccagccggcctctcgcccacactgaccccgggggagcggcagcagaaccggccctccgtgatcacctgtgcctcggctggcgcccgcaactgcaacctctcgcactgccccatcgcgcacagcggctgtgccgcgcccgggcctgccagctaccggaggccaccgagcgctgccaccacctgtgaccccgtggtggaggagcatttccgcaggagcctgggcaagaattacaaggagcccgagccggcacccaactccgtgtccatcacgggctccgtggacgaccactttgccaaagctctgggtgacacgtggctccagatcaaagcggccaaggacggagcatccagcagccctgagtccgcctctcgcaggggccagcccgccagcccctctgcccacatggtcagccacagtcactccccctctgtggtctccgccatggtgagcaagggcgaggagctgttcaccggggtggtgcccatcctggtcgagctggacggcgacgtaaacggccacaagttcagcgtgtccggcgagggcgagggcgatgccacctacggcaagctgaccctgaagttcatctgcaccaccggcaagctgcccgtgccctggcccaccctcgtgaccaccctgacctacggcgtgcagtgcttcagccgctaccccgaccacatgaagcagcacgacttcttcaagtccgccatgcccgaaggctacgtccaggagcgcaccatcttcttcaaggacgacggcaactacaagacccgcgccgaggtgaagttcgagggcgacaccctggtgaaccgcatcgagctgaagggcatcgacttcaaggaggacggcaacatcctggggcacaagctggagtacaactacaacagccacaacgtctatatcatggccgacaagcagaagaacggcatcaaggtgaacttcaagatccgccacaacatcgaggacggcagcgtgcagctcgccgaccactaccagcagaacacccccatcggcgacggccccgtgctgctgcccgacaaccactacctgagcacccagtccgccctgagcaaagaccccaacgagaagcgcgatcacatggtcctgctggagttcgtgaccgccgccgggatcactctcggcatggacgagctgtacaagtaa

SEQ ID NO: 40 - DNA, 2816 bp, Artificial Sequence
  Laboratory-synthesized seqeunce
gcatgccaatttatagtgccgtcactaacagtactgatactttaacatgctaagtttaaagtgtgtgctatattaattgtaagattggtgaagagaggtgttatcagatggaagctgcagcagcctggattaatgtggttaaatgtatcttctcctgtgattactgtctttatttcttcttttaaaatattgtcatttggacatctatctgtatagctacgccctgacacgtcctcctggagacagataagaagttacgacgggaggagcagatggaggcaaagcgctgtgatgcttttgtggtttgagtgcacacatttgttcagtgattctgtgaaatgagtgagcaaatggtgaccgggtgccctgtaaatggtgttctacatcttaagagaagaacacggacactaggtaagtgaagcttgctgtcactcctctacagcgtcacagagggtcagtcacccttgaccacactgaactagtcgtcacctttccactcttcctgccagaagagcagaaatcagactctctggggatatcagcctcacccctactgctctctccattatgaggcaaactttctttcacttcccagaggctctgggggcagcaaggtcaaccctttcctcagactctagtctcggaggagatcagatcgcgcttattcaagggaaccagcccctgctctgcgccctggtccaaggctgttgaagagtgacaaaaggcaccacgctgcggggacgcgggtgaagcccctctgtgtgtcctctgggcataatcaggaactggtgccaaatcagaggtgatgtggccagggctttgggagtgacgcgcggctgggaggcttgcgcacccaaggcacgcccctgccaagtcccactagcagctctttggagacctgggccggctcagccacttcccccagtccctcctccggcaaggggctatatagatctcccaggtcagggcgcagctgcagaagttggtcgtgaggcactgggcaggtaagtatcaaggttacaagacaggtttaaggagaccaatagaaactgggcttgtcgagacagagaagactcttgcgtttctgataggcacctattggtcttactgacatcgcagctgcctttctctccacaggtgtccactcccagttcaattacagctcttaaggctagagtacttaatacgactcactataggctagcatgctatttatgaagatggacctgttgaactatcagtacttggacaagatgaacaacaatatcggcattctgtgctacgaaggcgaagctgctctcaggggagaacccagaatgcagaccctgccggtggcctctgccctcagcagtcaccgcaccggccctcccccaatcagccccagcaagaggaagttcagcatggagccaggtgacgaggacctagactgtgacaacgaccacgtctccaaaatgagtcgcatcttcaacccccatctgaacaagactgccaatggagactgccgcagagacccccgggagcggagccgcagccccatcgagcgcgctgtggcccccaccatgagcctgcacggcagccacctgtacacctccctccccagccttggcctggagcagcccctcgcactgaccaagaacagcctggacgccagcaggccagccggcctctcgcccacactgaccccgggggagcggcagcagaaccggccctccgtgatcacctgtgcctcggctggcgcccgcaactgcaacctctcgcactgccccatcgcgcacagcggctgtgccgcgcccgggcctgccagctaccggaggccaccgagcgctgccaccacctgtgaccccgtggtggaggaggcagcccgcaggagcctgggcaagaattacaaggagcccgagccggcacccaactccgtgtccatcacgggctccgtggacgacgcagctgccaaagctctgggtgacacgtggctccagatcaaagcggccaaggacggagcatccagcagccctgagtccgcctctcgcaggggccagcccgccagcccctctgcccacatggtcagccacagtcactccccctctgtggtctccgccatggtgagcaagggcgaggagctgttcaccggggtggtgcccatcctggtcgagctggacggcgacgtaaacggccacaagttcagcgtgtccggcgagggcgagggcgatgccacctacggcaagctgaccctgaagttcatctgcaccaccggcaagctgcccgtgccctggcccaccctcgtgaccaccctgacctacggcgtgcagtgcttcagccgctaccccgaccacatgaagcagcacgacttcttcaagtccgccatgcccgaaggctacgtccaggagcgcaccatcttcttcaaggacgacggcaactacaagacccgcgccgaggtgaagttcgagggcgacaccctggtgaaccgcatcgagctgaagggcatcgacttcaaggaggacggcaacatcctggggcacaagctggagtacaactacaacagccacaacgtctatatcatggccgacaagcagaagaacggcatcaaggtgaacttcaagatccgccacaacatcgaggacggcagcgtgcagctcgccgaccactaccagcagaacacccccatcggcgacggccccgtgctgctgcccgacaaccactacctgagcacccagtccgccctgagcaaagaccccaacgagaagcgcgatcacatggtcctgctggagttcgtgaccgccgccgggatcactctcggcatggacgagctgtacaagtaa

SEQ ID NO: 41 - protein, 16 aa, Homo sapiens
DPVVEEHFRRSLGKNY

SEQ ID NO: 42 - protein, 16 aa, Homo sapiens
TGSVDDHFAKALGDTW

SEQ ID NO: 43 - protein, 16 aa, Artificial Sequence
  Homo sapiens
DPVVEEAARRSLGKNY

SEQ ID NO: 44 - protein, 16 aa, Artificial Sequence
  Homo sapiens
TGSVDDAAAKALGDTW